European Patent Application EP 4 130 294 A1, published February 8, 2023. Title: UNIVERSAL PROBE CHIP-BASED MULTIPLEX QUANTITATIVE PCR TESTING SYSTEM. Applicant: FLASHDX SHENZHEN INC. The sequence listing filed with the application follows.

SEQUENCE LISTING (14 sequences)

SEQ ID NO: 1 - DNA, 83 bp, artificial sequence
  a first primer
tgttgcgttctcaatgatacggcgaccaccgattaccatgcagaaggaggcaaagtaaggaggtttggactgagaacgcaaca

SEQ ID NO: 2 - DNA, 46 bp, artificial sequence
  a second primer
caagcagaagacggcatacgagatacaggctggctcaggactatct

SEQ ID NO: 3 - DNA, 20 bp, artificial sequence
  A fourth primer
aatgatacggcgaccaccga

SEQ ID NO: 4 - DNA, 24 bp, artificial sequence
  A fifth primer
caagcagaagacggcatacgagat

SEQ ID NO: 5 - DNA, 29 bp, artificial sequence
  A sixth probe
accatgcagaaggaggcaaagtaaggagg

SEQ ID NO: 6 - DNA, 29 bp, artificial sequence
  A seventh probe
cctccttactttgcctccttctgcatggt

SEQ ID NO: 7 - DNA, 111 bp, artificial sequence
  Target substrate 1
tttggactgagaacgcaacacatggaggttgctagtcaggccaggacaaatggtgcaggcaatgagagagccattgggactcatcccagagatagtcctgagccagcctgt

SEQ ID NO: 8 - DNA, 29 bp, artificial sequence
  Taqman probe for Target tradition
ggacaaatggtgcaggcaatgagagagag

SEQ ID NO: 9 - DNA, 40 bp, artificial sequence
  Forward
aatgatacggcgaccaccgatttggactgagaacgcaaca

SEQ ID NO: 10 - DNA, 79 bp, artificial sequence
  A first primer
cgatgccagttcaatgatacggcgaccaccgattccctcaacggtatcgcgtcggttgctgtgtactacactggcatcg

SEQ ID NO: 11 - DNA, 50 bp, artificial sequence
  A  second  primer
caagcagaagacggcatacgagatgtactcaggctgacagtaagtcttag

SEQ ID NO: 12 - DNA, 25 bp, artificial sequence
  Quenching (a sixth) probe
ccctcaacggtatcgcgtcggttgc

SEQ ID NO: 13 - DNA, 25 bp, artificial sequence
  Microarray Surface (a Seventh) Probe
gcaaccgacgcgataccgttgaggg

SEQ ID NO: 14 - DNA, 102 bp, artificial sequence
  Target substrate 2
tgtgtactacactggcatcgcatggagcactgatatcgccttcgaataacaattatacccgcgagaaatctttgagctaagacttactgtcagcctgagtac